European Patent Specification EP 3 259 358 B1, published June 19, 2024. Title: ENHANCED PROTEIN EXPRESSION. Applicant: Danisco. The sequence listing filed with the application follows.

SEQUENCE LISTING (26 sequences)

SEQ ID NO: 1 - DNA, 1726 bp, Artificial Sequence
  synthetic construct
ctcgaggcttttcttttggaagaaaatatagggaaaatggtacttgttaaaaattcggaatatttatacaatatcatatgtttcacattgaaaggggaggagaatcatgaaacaacaaaaacggctttacgcccgattgctgacgctgttatttgcgctcatcttcttgctgcctcattctgcagcttcagcagcaaatcttaatgggacgctgatgcagtattttgaatggtacatgcccaatgacggccaacattggaagcgtttgcaaaacgactcggcatatttggctgaacacggtattactgccgtctggattcccccggcatataagggaacgagccaagcggatgtgggctacggtgcttacgacctttatgatttaggggagtttcatcaaaaagggacggttcggacaaagtacggcacaaaaggagagctgcaatctgcgatcaaaagtcttcattcccgcgacattaacgtttacggggatgtggtcatcaaccacaaaggcggcgctgatgcgaccgaagatgtaaccgcggttgaagtcgatcccgctgaccgcaaccgcgtaatttcaggagaacacctaattaaagcctggacacattttcattttccggggcgcggcagcacatacagcgattttaaatggcattggtaccattttgacggaaccgattgggacgagtcccgaaagctgaaccgcatctataagtttcaaggaaaggcttgggattgggaagtttccaatgaaaacggcaactatgattatttgatgtatgccgacatcgattatgaccatcctgatgtcgcagcagaaattaagagatggggcacttggtatgccaatgaactgcaattggacggtttccgtcttgatgctgtcaaacacattaaattttcttttttgcgggattgggttaatcatgtcagggaaaaaacggggaaggaaatgtttacggtagctgaatattggcagaatgacttgggcgcgctggaaaactatttgaacaaaacaaattttaatcattcagtgtttgacgtgccgcttcattatcagttccatgctgcatcgacacagggaggcggctatgatatgaggaaattgctgaacggtacggtcgtttccaagcatccgttgaaatcggttacatttgtcgataaccatgatacacagccggggcaatcgcttgagtcgactgtccaaacatggtttaagccgcttgcttacgcttttattctcacaagggaatctggataccctcaggttttctacggggatatgtacgggacgaaaggagactcccagcgcgaaattcctgccttgaaacacaaaattgaaccgatcttaaaagcgagaaaacagtatgcgtacggagcacagcatgattatttcgaccaccatgacattgtcggctggacaagggaaggcgacagctcggttgcaaattcaggtttggcggcattaataacagacggacccggtggggcaaagcgaatgtatgtcggccggcaaaacgccggtgagacatggcatgacattaccggaaaccgttcggagccggttgtcatcaattcggaaggctggggagagtttcacgtaaacggcgggtcggtttcaatttatgttcaaagatgagttaacagaggacggatttcctgaaggaaatccgtttttttattttaagcttggagacaaggtaaaggataaaacctcgag

SEQ ID NO: 2 - DNA, 59 bp, Artificial Sequence
  synthetic construct
gacagaatagtcttttaagtaagtctactctgaatttttttaaaaggagagggtaaaga

SEQ ID NO: 3 - DNA, 1764 bp, Artificial Sequence
  synthetic construct
ctcgaggcttttcttttggaagaaaatatagggaaaatggtacttgttaaaaattcggaatatttatacaatatcatatgacagaatagtcttttaagtaagtctactctgaatttttttaaaaggagagggtaaagaatgaaacaacaaaaacggctttacgcccgattgctgacgctgttatttgcgctcatcttcttgctgcctcattctgcagcttcagcagcaaatcttaatgggacgctgatgcagtattttgaatggtacatgcccaatgacggccaacattggaagcgtttgcaaaacgactcggcatatttggctgaacacggtattactgccgtctggattcccccggcatataagggaacgagccaagcggatgtgggctacggtgcttacgacctttatgatttaggggagtttcatcaaaaagggacggttcggacaaagtacggcacaaaaggagagctgcaatctgcgatcaaaagtcttcattcccgcgacattaacgtttacggggatgtggtcatcaaccacaaaggcggcgctgatgcgaccgaagatgtaaccgcggttgaagtcgatcccgctgaccgcaaccgcgtaatttcaggagaacacctaattaaagcctggacacattttcattttccggggcgcggcagcacatacagcgattttaaatggcattggtaccattttgacggaaccgattgggacgagtcccgaaagctgaaccgcatctataagtttcaaggaaaggcttgggattgggaagtttccaatgaaaacggcaactatgattatttgatgtatgccgacatcgattatgaccatcctgatgtcgcagcagaaattaagagatggggcacttggtatgccaatgaactgcaattggacggtttccgtcttgatgctgtcaaacacattaaattttcttttttgcgggattgggttaatcatgtcagggaaaaaacggggaaggaaatgtttacggtagctgaatattggcagaatgacttgggcgcgctggaaaactatttgaacaaaacaaattttaatcattcagtgtttgacgtgccgcttcattatcagttccatgctgcatcgacacagggaggcggctatgatatgaggaaattgctgaacggtacggtcgtttccaagcatccgttgaaatcggttacatttgtcgataaccatgatacacagccggggcaatcgcttgagtcgactgtccaaacatggtttaagccgcttgcttacgcttttattctcacaagggaatctggataccctcaggttttctacggggatatgtacgggacgaaaggagactcccagcgcgaaattcctgccttgaaacacaaaattgaaccgatcttaaaagcgagaaaacagtatgcgtacggagcacagcatgattatttcgaccaccatgacattgtcggctggacaagggaaggcgacagctcggttgcaaattcaggtttggcggcattaataacagacggacccggtggggcaaagcgaatgtatgtcggccggcaaaacgccggtgagacatggcatgacattaccggaaaccgttcggagccggttgtcatcaattcggaaggctggggagagtttcacgtaaacggcgggtcggtttcaatttatgttcaaagatgagttaacagaggacggatttcctgaaggaaatccgtttttttattttaagcttggagacaaggtaaaggataaaacagctgcggccgc

SEQ ID NO: 4 - DNA, 34 bp, Artificial Sequence
  primer
cggtttagcagctgcgctagctgcagaatgaggc

SEQ ID NO: 5 - DNA, 35 bp, Artificial Sequence
  primer
cggcaaaaaatgaaagcttctcgaggttaacagag

SEQ ID NO: 6 - DNA, 35 bp, Artificial Sequence
  synthetic
cagctagcgcagctgctaaaccggcagtcagcaac

SEQ ID NO: 7 - DNA, 35 bp, Artificial Sequence
  primer
cgagaagctttcattttttgccgtggtccgggctg

SEQ ID NO: 8 - DNA, 26 bp, Artificial Sequence
  synthetic
gtttcacattgaaaggggaggagaat

SEQ ID NO: 9 - DNA, 59 bp, Artificial Sequence
  synthetic
gaccgcatagtccgttaagtgggtctacgcggaatttttttaaaaggagagggtaaaga

SEQ ID NO: 10 - DNA, 63 bp, Artificial Sequence
  synthetic
gacagaatagtcttttaagtaagtctactctgtttcacattgaaaggaaaggagagggtaatc

SEQ ID NO: 11 - DNA, 2787 bp, Artificial Sequence
  synthetic construct
ctcgaggcttttcttttggaagaaaatatagggaaaatggtacttgttaaaaattcggaatatttatacaatatcatatgacagaatagtcttttaagtaagtctactctgaatttttttaaaaggagagggtaaagaatgaaacaacaaaaacggctttacgcccgattgctgacgctgttatttgcgctcatcttcttgctgcctcattctgcagcttcagcagctgctaaaccggcagtcagcaacgcttatctggatgccagcaaccaagtcctggtcaaactgagccaaccgctgacacttggagaaggagcgagcggatttacggtccatgatgacacggcgaacaaagatatcccggtcacgagcgttaaagatgctagcctgggccaagatgtcacagcagttctggcgggcacgtttcaacatatctttggcggatcagattgggcaccggataatcacagcacgctgctgaaaaaagtcacgaacaacctgtatcagtttagcggagatctgccggaaggcaactatcaatataaagtcgccctgaacgatagctggaacaatccgagctatccgagcgataacatcaatctgacagtcccggcaggcggagcacatgtcacgtttagctatatcccgagcacacatgccgtctatgacacgatcaacaacccgaacgccgatcttcaagtcgaaagcggcgtcaaaacggatctggtcacagtcacattgggagaagatccggatgtcagccatacactgagcatccaaacggatggctatcaagcgaaacaagtcatcccgagaaacgtcctgaacagcagccagtattattatagcggcgatgatctgggcaacacgtatacacaaaaagcgacgacgtttaaagtttgggcgccgacaagcacacaagtcaacgtcctgctgtatgattcagcaacaggcagcgtcacaaaaatcgtcccgatgacagcatcaggacatggagtctgggaagcgacggtcaaccaaaacctggaaaactggtattatatgtatgaagtcacgggccaaggatcaacaagaacagcggtcgatccgtatgctacagcaatcgccccgaatggaacaagaggcatgatcgtcgatctggcaaaaacagacccggcaggctggaatagcgataaacatatcacgccgaaaaacatcgaagatgaagtcatctatgaaatggacgtccgggattttagcatcgatccgaacagcggcatgaaaaacaaaggcaaatatctggcgctgacggaaaaaggaacaaaaggcccggataacgtcaaaacaggcatcgatagcctgaaacaactgggcatcacacatgtccaactgatgccggtctttgctagcaatagcgtcgatgaaacggacccgacacaagataactggggctatgacccgagaaattatgatgtcccggaaggccaatatgccacgaacgccaatggaaacgcccggatcaaagaatttaaagaaatggtcctgagccttcatagagaacatatcggcgtcaacatggacgtcgtctataaccatacgtttgccacacagatcagcgactttgataaaatcgtgccggaatattattatcggacggatgacgccggcaattatacgaatggcagcggcacaggaaatgaaatcgccgccgaaagaccgatggtccagaaatttatcatcgacagccttaaatattgggtcaacgaatatcatatcgacggctttcgctttgatctgatggcgctgctgggcaaagatacaatgagcaaagcggcgagcgaacttcatgctatcaatccgggcatcgctctttatggagaaccgtggacaggaggaacatcagcactgccggatgatcaactgctgacaaaaggcgcccaaaaaggaatgggagtcgccgtctttaacgacaacctgagaaatgccctggatggcaacgtttttgatagcagcgcccaaggatttgctacaggagcgacaggactgacagatgccatcaaaaatggcgtcgaaggcagcatcaacgattttacaagcagcccgggagagacgatcaattatgtcacgagccatgacaactatacgctgtgggacaaaatcgctctgagcaacccgaatgatagcgaagcggaccggatcaaaatggatgaactggcacaagcagtcgtcatgacatcacaaggcgtcccgtttatgcaaggcggagaagaaatgctgagaacgaaaggcggcaacgacaacagctataatgccggcgatgccgtcaatgaatttgactggagccggaaagcacaatatccggacgtctttaactattattcaggacttatccatctgagactggaccatccggcgtttagaatgacgacggcgaacgaaatcaacagccatcttcagtttctgaacagcccggaaaatacggtcgcctatgaactgacggaccatgtgaacaaagacaaatggggcaacatcatcgtcgtttataacccgaacaaaacggtcgccacaatcaatcttccgagcggcaaatgggcaatcaatgccacaagcggcaaagttggagaaagcacactgggacaagcagaaggatcagtccaagtcccgggaatcagcatgatgatccttcatcaagaagtcagcccggaccacggcaaaaaataagttaacagaggacggatttcctgaaggaaatccgtttttttattttaagcttggagacaaggtaaaggataaaacagctgcggccgc

SEQ ID NO: 12 - DNA, 1777 bp, Artificial Sequence
  synthetic construct
tcgctgataaacagctgacatcaactaaaagcttcattaaatactttgaaaaaagttgttgacttaaaagaagctaaatgttatagtaataaaacagaatagtcttttaagtaagtctactctgaatttttttaaaaggagagggtaaagaatgaaacaacaaaaacggctttacgcccgattgctgacgctgttatttgcgctcatcttcttgctgcctcattctgcagctagcgcagcaaatcttaatgggacgctgatgcagtattttgaatggtacatgcccaatgacggccaacattggaagcgtttgcaaaacgactcggcatatttggctgaacacggtattactgccgtctggattcccccggcatataagggaacgagccaagcggatgtgggctacggtgcttacgacctttatgatttaggggagtttcatcaaaaagggacggttcggacaaagtacggcacaaaaggagagctgcaatctgcgatcaaaagtcttcattcccgcgacattaacgtttacggggatgtggtcatcaaccacaaaggcggcgctgatgcgaccgaagatgtaaccgcggttgaagtcgatcccgctgaccgcaaccgcgtaatttcaggagaacacctaattaaagcctggacacattttcattttccggggcgcggcagcacatacagcgattttaaatggcattggtaccattttgacggaaccgattgggacgagtcccgaaagctgaaccgcatctataagtttcaaggaaaggcttgggattgggaagtttccaatgaaaacggcaactatgattatttgatgtatgccgacatcgattatgaccatcctgatgtcgcagcagaaattaagagatggggcacttggtatgccaatgaactgcaattggacggtttccgtcttgatgctgtcaaacacattaaattttcttttttgcgggattgggttaatcatgtcagggaaaaaacggggaaggaaatgtttacggtagctgaatattggcagaatgacttgggcgcgctggaaaactatttgaacaaaacaaattttaatcattcagtgtttgacgtgccgcttcattatcagttccatgctgcatcgacacagggaggcggctatgatatgaggaaattgctgaacggtacggtcgtttccaagcatccgttgaaatcggttacatttgtcgataaccatgatacacagccggggcaatcgcttgagtcgactgtccaaacatggtttaagccgcttgcttacgcttttattctcacaagggaatctggataccctcaggttttctacggggatatgtacgggacgaaaggagactcccagcgcgaaattcctgccttgaaacacaaaattgaaccgatcttaaaagcgagaaaacagtatgcgtacggagcacagcatgattatttcgaccaccatgacattgtcggctggacaagggaaggcgacagctcggttgcaaattcaggtttggcggcattaataacagacggacccggtggggcaaagcgaatgtatgtcggccggcaaaacgccggtgagacatggcatgacattaccggaaaccgttcggagccggttgtcatcaattcggaaggctggggagagtttcacgtaaacggcgggtcggtttcaatttatgttcaaagatgagttaacagaggacggatttcctgaaggaaatccgtttttttattttaagcttggagacaaggtaaaggataaaacagctgcggccgc

SEQ ID NO: 13 - DNA, 2890 bp, Artificial Sequence
  synthetic construct
tcgctgataaacagctgacatcaactaaaagcttcattaaatactttgaaaaaagttgttgacttaaaagaagctaaatgttatagtaataaaacagaatagtcttttaagtaagtctactctgaatttttttaaaaggagagggtaaagaatgaaacaacaaaaacggctttacgcccgattgctgacgctgttatttgcgctcatcttcttgctgcctcattctgcagctagcgcagctgctaaaccggcagtcagcaacgcttatctggatgccagcaaccaagtcctggtcaaactgagccaaccgctgacacttggagaaggagcgagcggatttacggtccatgatgacacggcgaacaaagatatcccggtcacgagcgttaaagatgctagcctgggccaagatgtcacagcagttctggcgggcacgtttcaacatatctttggcggatcagattgggcaccggataatcacagcacgctgctgaaaaaagtcacgaacaacctgtatcagtttagcggagatctgccggaaggcaactatcaatataaagtcgccctgaacgatagctggaacaatccgagctatccgagcgataacatcaatctgacagtcccggcaggcggagcacatgtcacgtttagctatatcccgagcacacatgccgtctatgacacgatcaacaacccgaacgccgatcttcaagtcgaaagcggcgtcaaaacggatctggtcacagtcacattgggagaagatccggatgtcagccatacactgagcatccaaacggatggctatcaagcgaaacaagtcatcccgagaaacgtcctgaacagcagccagtattattatagcggcgatgatctgggcaacacgtatacacaaaaagcgacgacgtttaaagtttgggcgccgacaagcacacaagtcaacgtcctgctgtatgattcagcaacaggcagcgtcacaaaaatcgtcccgatgacagcatcaggacatggagtctgggaagcgacggtcaaccaaaacctggaaaactggtattatatgtatgaagtcacgggccaaggatcaacaagaacagcggtcgatccgtatgctacagcaatcgccccgaatggaacaagaggcatgatcgtcgatctggcaaaaacagacccggcaggctggaatagcgataaacatatcacgccgaaaaacatcgaagatgaagtcatctatgaaatggacgtccgggattttagcatcgatccgaacagcggcatgaaaaacaaaggcaaatatctggcgctgacggaaaaaggaacaaaaggcccggataacgtcaaaacaggcatcgatagcctgaaacaactgggcatcacacatgtccaactgatgccggtctttgctagcaatagcgtcgatgaaacggacccgacacaagataactggggctatgacccgagaaattatgatgtcccggaaggccaatatgccacgaacgccaatggaaacgcccggatcaaagaatttaaagaaatggtcctgagccttcatagagaacatatcggcgtcaacatggacgtcgtctataaccatacgtttgccacacagatcagcgactttgataaaatcgtgccggaatattattatcggacggatgacgccggcaattatacgaatggcagcggcacaggaaatgaaatcgccgccgaaagaccgatggtccagaaatttatcatcgacagccttaaatattgggtcaacgaatatcatatcgacggctttcgctttgatctgatggcgctgctgggcaaagatacaatgagcaaagcggcgagcgaacttcatgctatcaatccgggcatcgctctttatggagaaccgtggacaggaggaacatcagcactgccggatgatcaactgctgacaaaaggcgcccaaaaaggaatgggagtcgccgtctttaacgacaacctgagaaatgccctggatggcaacgtttttgatagcagcgcccaaggatttgctacaggagcgacaggactgacagatgccatcaaaaatggcgtcgaaggcagcatcaacgattttacaagcagcccgggagagacgatcaattatgtcacgagccatgacaactatacgctgtgggacaaaatcgctctgagcaacccgaatgatagcgaagcggaccggatcaaaatggatgaactggcacaagcagtcgtcatgacatcacaaggcgtcccgtttatgcaaggcggagaagaaatgctgagaacgaaaggcggcaacgacaacagctataatgccggcgatgccgtcaatgaatttgactggagccggaaagcacaatatccggacgtctttaactattattcaggacttatccatctgagactggaccatccggcgtttagaatgacgacggcgaacgaaatcaacagccatcttcagtttctgaacagcccggaaaatacggtcgcctatgaactgacggaccatgtgaacaaagacaaatggggcaacatcatcgtcgtttataacccgaacaaaacggtcgccacaatcaatcttccgagcggcaaatgggcaatcaatgccacaagcggcaaagttggagaaagcacactgggacaagcagaaggatcagtccaagtcccgggaatcagcatgatgatccttcatcaagaagtcagcccggaccacggcaaaaaataagttaacagaggacggatttcctgaaggaaatccgtttttttattttaagcttggagacaaggtaaaggataaaacagctgcggccgctgagttaacagaggacggatttcctgaaggaaatccgtttttttattttaagcttggagacaaggtaaaggataaaacagctgcggccgc

SEQ ID NO: 14 - DNA, 1726 bp, Artificial Sequence
  synthetic construct
gcttttcttttggaagaaaatatagggaaaatggtacttgttaaaaattcggaatatttatacaatatcatatgacagaatagtcttttaagtaagtctactctgaatttttttaaaaggagagggtaaagaatgaaacaacaaaaacggctttacgcccgattgctgacgctgttatttgcgctcatcttcttgctgcctcattctgcagcttcagcagccgcaccgtttaacggtaccatgatgcagtattttgaatggtacttgccggatgatggcacgttatggaccaaagtggccaatgaagccaacaacttatccagccttggcatcaccgctctttggctgccgcccgcttacaaaggaacaagccgcagcgacgtagggtacggagtatacgacttgtatgacctcggcgaattcaatcaaaaagggaccgtccgcacaaaatatggaacaaaagctcaatatcttcaagccattcaagccgcccacgccgctggaatgcaagtgtacgccgatgtcgtgttcgaccataaaggcggcgctgacggcacggaatgggtggacgccgtcgaagtcaatccgtccgaccgcaaccaagaaatctcgggcacctatcaaatccaagcatggacgaaatttgattttcccgggcggggcaacacctactccagctttaagtggcgctggtaccattttgacggcgttgattgggacgaaagccgaaaattaagccgcatttacaaattcaggggcatcggcaaagcgtgggattggccggtagacacagaaaacggaaactatgactacttaatgtatgccgaccttgatatggatcatcccgaagtcgtgaccgagctgaaaaactgggggaaatggtatgtcaacacaacgaacattgatgggttccggcttgatgccgtcaagcatattaagttcagtttttttcctgattggttgtcgtatgtgcgttctcagactggcaagccgctatttaccgtcggggaatattggagctatgacatcaacaagttgcacaattacattacgaaaacaaacggaacgatgtctttgtttgatgccccgttacacaacaaattttataccgcttccaaatcagggggcgcatttgatatgcgcacgttaatgaccaatactctcatgaaagatcaaccgacattggccgtcaccttcgttgataatcatgacaccgaacccggccaagcgcttcagtcatgggtcgacccatggttcaaaccgttggcttacgcctttattctaactcggcaggaaggatacccgtgcgtcttttatggtgactattatggcattccacaatataacattccttcgctgaaaagcaaaatcgatccgctcctcatcgcgcgcagggattatgcttacggaacgcaacatgattatcttgatcactccgacatcatcgggtggacaagggaaggggtcactgaaaaaccaggatccgggctggccgcactgatcaccgatgggccgggaggaagcaaatggatgtacgttggcaaacaacacgctggaaaagtgttctatgaccttaccggcaaccggagtgacaccgtcaccatcaacagtgatggatggggggaattcaaagtcaatggcggttcggtttcggtttgggttcctagaaaaacgacctgagttaacagaggacggatttcctgaaggaaatccgtttttttatttt

SEQ ID NO: 15 - DNA, 1726 bp, Artificial Sequence
  synthetic construct
gcttttcttttggaagaaaatatagggaaaatggtacttgttaaaaattcggaatatttatacaatatcatatgaccgcatagtccgttaagtgggtctacgcggaatttttttaaaaggagagggtaaagaatgaaacaacaaaaacggctttacgcccgattgctgacgctgttatttgcgctcatcttcttgctgcctcattctgcagcttcagcagccgcaccgtttaacggtaccatgatgcagtattttgaatggtacttgccggatgatggcacgttatggaccaaagtggccaatgaagccaacaacttatccagccttggcatcaccgctctttggctgccgcccgcttacaaaggaacaagccgcagcgacgtagggtacggagtatacgacttgtatgacctcggcgaattcaatcaaaaagggaccgtccgcacaaaatatggaacaaaagctcaatatcttcaagccattcaagccgcccacgccgctggaatgcaagtgtacgccgatgtcgtgttcgaccataaaggcggcgctgacggcacggaatgggtggacgccgtcgaagtcaatccgtccgaccgcaaccaagaaatctcgggcacctatcaaatccaagcatggacgaaatttgattttcccgggcggggcaacacctactccagctttaagtggcgctggtaccattttgacggcgttgattgggacgaaagccgaaaattaagccgcatttacaaattcaggggcatcggcaaagcgtgggattggccggtagacacagaaaacggaaactatgactacttaatgtatgccgaccttgatatggatcatcccgaagtcgtgaccgagctgaaaaactgggggaaatggtatgtcaacacaacgaacattgatgggttccggcttgatgccgtcaagcatattaagttcagtttttttcctgattggttgtcgtatgtgcgttctcagactggcaagccgctatttaccgtcggggaatattggagctatgacatcaacaagttgcacaattacattacgaaaacaaacggaacgatgtctttgtttgatgccccgttacacaacaaattttataccgcttccaaatcagggggcgcatttgatatgcgcacgttaatgaccaatactctcatgaaagatcaaccgacattggccgtcaccttcgttgataatcatgacaccgaacccggccaagcgcttcagtcatgggtcgacccatggttcaaaccgttggcttacgcctttattctaactcggcaggaaggatacccgtgcgtcttttatggtgactattatggcattccacaatataacattccttcgctgaaaagcaaaatcgatccgctcctcatcgcgcgcagggattatgcttacggaacgcaacatgattatcttgatcactccgacatcatcgggtggacaagggaaggggtcactgaaaaaccaggatccgggctggccgcactgatcaccgatgggccgggaggaagcaaatggatgtacgttggcaaacaacacgctggaaaagtgttctatgaccttaccggcaaccggagtgacaccgtcaccatcaacagtgatggatggggggaattcaaagtcaatggcggttcggtttcggtttgggttcctagaaaaacgacctgagttaacagaggacggatttcctgaaggaaatccgtttttttatttt

SEQ ID NO: 16 - DNA, 1730 bp, Artificial Sequence
  synthetic construct
gcttttcttttggaagaaaatatagggaaaatggtacttgttaaaaattcggaatatttatacaatatcatatgacagaatagtcttttaagtaagtctactctgtttcacattgaaaggaaaggagagggtaatcatgaaacaacaaaaacggctttacgcccgattgctgacgctgttatttgcgctcatcttcttgctgcctcattctgcagcttcagcagccgcaccgtttaacggtaccatgatgcagtattttgaatggtacttgccggatgatggcacgttatggaccaaagtggccaatgaagccaacaacttatccagccttggcatcaccgctctttggctgccgcccgcttacaaaggaacaagccgcagcgacgtagggtacggagtatacgacttgtatgacctcggcgaattcaatcaaaaagggaccgtccgcacaaaatatggaacaaaagctcaatatcttcaagccattcaagccgcccacgccgctggaatgcaagtgtacgccgatgtcgtgttcgaccataaaggcggcgctgacggcacggaatgggtggacgccgtcgaagtcaatccgtccgaccgcaaccaagaaatctcgggcacctatcaaatccaagcatggacgaaatttgattttcccgggcggggcaacacctactccagctttaagtggcgctggtaccattttgacggcgttgattgggacgaaagccgaaaattaagccgcatttacaaattcaggggcatcggcaaagcgtgggattggccggtagacacagaaaacggaaactatgactacttaatgtatgccgaccttgatatggatcatcccgaagtcgtgaccgagctgaaaaactgggggaaatggtatgtcaacacaacgaacattgatgggttccggcttgatgccgtcaagcatattaagttcagtttttttcctgattggttgtcgtatgtgcgttctcagactggcaagccgctatttaccgtcggggaatattggagctatgacatcaacaagttgcacaattacattacgaaaacaaacggaacgatgtctttgtttgatgccccgttacacaacaaattttataccgcttccaaatcagggggcgcatttgatatgcgcacgttaatgaccaatactctcatgaaagatcaaccgacattggccgtcaccttcgttgataatcatgacaccgaacccggccaagcgcttcagtcatgggtcgacccatggttcaaaccgttggcttacgcctttattctaactcggcaggaaggatacccgtgcgtcttttatggtgactattatggcattccacaatataacattccttcgctgaaaagcaaaatcgatccgctcctcatcgcgcgcagggattatgcttacggaacgcaacatgattatcttgatcactccgacatcatcgggtggacaagggaaggggtcactgaaaaaccaggatccgggctggccgcactgatcaccgatgggccgggaggaagcaaatggatgtacgttggcaaacaacacgctggaaaagtgttctatgaccttaccggcaaccggagtgacaccgtcaccatcaacagtgatggatggggggaattcaaagtcaatggcggttcggtttcggtttgggttcctagaaaaacgacctgagttaacagaggacggatttcctgaaggaaatccgtttttttatttt

SEQ ID NO: 17 - DNA, 58 bp, Artificial Sequence
  synthetic
acagaatagtcttttaagtaagtctactctgaatttttttaaaaggagagggtaaaga

SEQ ID NO: 18 - DNA, 65 bp, Artificial Sequence
  synthetic
atagattttttttaaaaaactattgcaataaataaatacaggtgttatattattaaacgtcgctg

SEQ ID NO: 19 - DNA, 66 bp, Artificial Sequence
  synthetic
cacatacagcctaaattgggtgttgaccttttgataatatccgtgatatattattattcgtcgctg

SEQ ID NO: 20 - DNA, 64 bp, Artificial Sequence
  synthetic
ttaaatactttgaaaaaagttgttgacttaaaagaagctaaatgttatagtaataaagctgctt

SEQ ID NO: 21 - DNA, 65 bp, Artificial Sequence
  synthetic
ataaaaaaatacaggaaaagtgttgaccaaataaaacaggcatggtatattattaaacgtcgctg

SEQ ID NO: 22 - DNA, 65 bp, Artificial Sequence
  synthetic
aacaaaaaagttttcctaaggtgtttacaagattttaaaaatgtgtataataagaaaagtcgaat

SEQ ID NO: 23 - DNA, 64 bp, Artificial Sequence
  synthetic
tcgaaaaaacattaaaaaacttcttgactcaacatcaaatgatagtatgatagttaagtcgctc

SEQ ID NO: 24 - DNA, 112 bp, Artificial Sequence
  synthetic
gtttttatcacctaaaagtttaccactaatttttgtttattatatcataaacggtgaagcaataatggaggaatggttgacttcaaaacaaataaattatataatgaccttt

SEQ ID NO: 25 - DNA, 303 bp, Artificial Sequence
  synthetic
gtaccgtgtgttttcatttcagggaaacatgacttaattgttcctgcagaaatatcgaaacagtattatcaagaacttgaggcacctgaaaagcgctggtttcaatttgagaattcagctcacaccccgcatattgaggagccatcattattcgcgaacacattaagtcggcatgcacgcaaccatttatgatagatccttgataaataagaaaaacccctgtataataaaaaaagtgtgcaaatgatgcatattttaaataagtcttgcaacatgcgcctattttctgtataatggtgtata

SEQ ID NO: 26 - DNA, 103 bp, Artificial Sequence
  synthetic
aacatataactcaggacgctctatcctgggtttttggctgtgccaaaagggaataatgaaaaacaatagcatctttgtgaagtttgtattataataaaaaatt